European Patent Specification EP 3 856 156 B1, published October 29, 2025. Title: TREATMENT PF DEMENTIA-ASSOCIATED TAUOPATHIES. Applicant: Medizinische Hochschule Hannover (MHH), Deutsches Zentrum für Neurodegenerative Erkrankungen. The sequence listing filed with the application follows.

SEQUENCE LISTING (8 sequences)

SEQ ID NO: 1 - DNA, 19 bp, Artificial sequence
  Target sequence for short hairpins_1
actaccgttgttataggtg

SEQ ID NO: 2 - DNA, 19 bp, Artificial sequence
  Target sequence for short hairpins_2
tcctttatcattatggtgt

SEQ ID NO: 3 - DNA, 20 bp, Artificial sequence
  GAPDH_forward primer
tgcaccaccaactgcttagc

SEQ ID NO: 4 - DNA, 21 bp, Artificial sequence
  GAPDH_reverse primer
ggcatggactgtggtcatgag

SEQ ID NO: 5 - DNA, 26 bp, Artificial sequence
  probe_1
ccctggccaaggtcatccatgacaac

SEQ ID NO: 6 - DNA, 24 bp, Artificial sequence
  WPRE_forward primer
cctggttgctgtctctttatgagg

SEQ ID NO: 7 - DNA, 19 bp, Artificial sequence
  WPRE_reverse primer
tgacaggtggtggcaatgc

SEQ ID NO: 8 - DNA, 25 bp, Artificial sequence
  probe_2
cgttgtcaggcaacgtggcgtggtg